European Patent Specification EP 3 645 038 B1, published February 18, 2026. Title: GENETICALLY-MODIFIED T CELLS COMPRISING A MODIFIED INTRON IN THE T CELL RECEPTOR ALPHA GENE. Applicant: Jantz, Derek Smith, James J Beard, Clayton. The sequence listing filed with the application follows.

SEQUENCE LISTING (66 sequences)

SEQ ID NO: 1 - protein, 163 aa, Chlamydomonas reinhardtii
MNTKYNKEFLLYLAGFVDGDGSIIAQIKPNQSYKFKHQLSLAFQVTQKTQRRWFLDKLVDEIGVGYVRDRGSVSDYILSEIKPLHNFLTQLQPFLKLKQKQANLVLKIIWRLPSAKESPDKFLEVCTWVDQIAALNDSKTRKTTSETVRAVLDSLSEKKKSSP

SEQ ID NO: 2 - protein, 9 aa, Chlamydomonas reinhardtii
LAGLIDADG

SEQ ID NO: 3 - DNA, 577 bp, Homo sapiens
tgctgtgacttgctcaaggccttatatcaagtaaacggtagcgctggggcttagacgcaggtgttctgatttatagttcaaaacctctatcaatgagagagcaatctcctggtaatgtgatagatttcccaacttaatgccaacataccataaacctcccattctgctaatgcccagcctaagttggggagaccactccagattccaagatgtacagtttgctttgctgggcctttttcccatgcctgcctttactctgccagagttatattgctggggttttgaagaagatcctattaaataaaagaataagcagtattattaagtagccctgcatttcaggtttccttgagtggcaggccaggcctggccgtgaacgttcactgaaatcatggcctcttggccaagattgatagcttgtgcctgtccctgagtcccagtccatcacgagcagctggtttctaagatgctatttcccgtataaagcatgagaccgtgacttgccagccccacagagccccgcccttgtccatcactggcatctggactccagcctgggttggggcaaagagggaaa

SEQ ID NO: 4 - DNA, 22 bp, Homo sapiens
tgatagcttgtgcctgtccctg

SEQ ID NO: 5 - DNA, 22 bp, Homo sapiens
actatcgaacacggacagggac

SEQ ID NO: 6 - DNA, 22 bp, Homo sapiens
cagtttgctttgctgggccttt

SEQ ID NO: 7 - DNA, 22 bp, Homo sapiens
gtcaaacgaaacgacccggaaa

SEQ ID NO: 8 - DNA, 22 bp, Homo sapiens
tgctgtgacttgctcaaggcct

SEQ ID NO: 9 - DNA, 22 bp, Homo sapiens
acgacactgaacgagttccgga

SEQ ID NO: 10 - DNA, 22 bp, Homo sapiens
tgggttggggcaaagagggaaa

SEQ ID NO: 11 - DNA, 22 bp, Homo sapiens
acccaaccccgtttctcccttt

SEQ ID NO: 12 - protein, 354 aa, Artificial Sequence
  Synthesized
MNTKYNKEFLLYLAGFVDGDGSIFATIQPSQHRKFKHQLVLWFRVTQKTQRRWFLDKLVDEIGVGYVRDTGSVSYYSLSQIKPLHNFLTQLQPFLKLKQKQANLVLKIIEQLPSAKESPDKFLEVCTWVDQIAALNDSKTRKTTSETVRAVLDSLPGSVGGLSPSQASSAASSASSSPGSGISEALRAGAGSGTGYNKEFLLYLAGFVDGDGSIYATINPVQWNKFKHQLRLTFAVTQKTQRRWFLDKLVDEIGVGYVSDWGSVSQYKLSEIKPLHNFLTQLQPFLKLKQKQANLVLKIIEQLPSAKESPDKFLEVCTWVDQIAALNDSKTRKTTSETVRAVLDSLSEKKKSSP

SEQ ID NO: 13 - protein, 354 aa, Artificial Sequence
  Synthesized
MNTKYNKEFLLYLAGFVDGDGSIYATIRPDQVRKFKHQLTLYFRVSQKTQRRWFLDKLVDEIGVGYVNDCGSVSHYSLSQIKPLHNFLTQLQPFLKLKQKQANLVLKIIEQLPSAKESPDKFLEVCTWVDQIAALNDSKTRKTTSETVRAVLDSLPGSVGGLSPSQASSAASSASSSPGSGISEALRAGAGSGTGYNKEFLLYLAGFVDGDGSIFATIDPEQTGKFKHKLRLRFVVTQKTQRRWFLDKLVDEIGVGYVTDWGSVSYYRLSEIKPLHNFLTQLQPFLKLKQKQANLVLKIIEQLPSAKESPDKFLEVCTWVDQIAALNDSKTRKTTSETVRAVLDSLSEKKKSSP

SEQ ID NO: 14 - protein, 354 aa, Artificial Sequence
  Synthesized
MNTKYNKEFLLYLAGFVDGDGSIFATIQPSQHRKFKHQLVLWFRVTQKTQRRWFLDKLVDEIGVGYVRDTGSVSYYSLSKIKPLHNFLTQLQPFLKLKQKQANLVLKIIEQLPSAKESPDKFLEVCTWVDQIAALNDSKTRKTTSETVRAVLDSSPGSVGGLSPSQASSAASSASSSPGSGISEALRAGAGSGTGYNKEFLLYLAGFVDGDGSIFASIEPIQYSKFKHRLKLYFAVSQKTQRRWFLDKLVDEIGVGYVTDHGSVSTYRLSKIKPLHNFLTQLQPFLKLKQKQANLVLKIIEQLPSAKESPDKFLEVCTWVDQIAALNDSKTRKTTSETVRAVLDSLSEKKKSSP

SEQ ID NO: 15 - protein, 354 aa, Artificial Sequence
  Synthesized
MNTKYNKEFLLYLAGFVDGDGSIYATIQPGQTRKFKHQLSLWFRVTQKTQRRWFLDKLVDEIGVGYVSDAGSVSHYSLSQIKPLHNFLTQLQPFLKLKQKQANLVLKIIEQLPSAKESPDKFLEVCTWVDQIAALNDSKTRKTTSETVRAVLDSLPGSVGGLSPSQASSAASSASSSPGSGISEALRAGAGSGTGYNKEFLLYLAGFVDGDGSIYAAIEPTQCAKFKHKLRLLFAVTQKTQRRWFLDKLVDEIGVGYVYDQGSVSTYRLSQIKPLHNFLTQLQPFLKLKQKQANLVLKIIEQLPSAKESPDKFLEVCTWVDQIAALNDSKTRKTTSETVRAVLDSLSEKKKSSP

SEQ ID NO: 16 - protein, 354 aa, Artificial Sequence
  Synthesized
MNTKYNKEFLLYLAGFVDGDGSIHATIVPSQQYKFKHRLHLFFGVYQKTQRRWFLDKLVDEIGVGYVYDGGSVSRYILSEIKPLHNFLTQLQPFLKLKQKQANLVLKIIEQLPSAKESPDKFLEVCTWVDQIAALNDSKTRKTTSETVRAVLDSLPGSVGGLSPSQASSAASSASSSPGSGISEALRAGAGSGTGYNKEFLLYLAGFVDGDGSIYARILPVQVAKFKHQLRLTFRVGQKTQRRWFLDKLVDEIGVGYVSDSGSVSNYELSQIKPLHNFLTQLQPFLKLKQKQANLVLKIIEQLPSAKESPDKFLEVCTWVDQIAALNDSKTRKTTSETVRAVLDSLSEKKKSSP

SEQ ID NO: 17 - protein, 354 aa, Artificial Sequence
  Synthesized
MNTKYNKEFLLYLAGFVDGDGSIHATIVPSQQYKFKHRLHLFFGVYQKTQRRWFLDKLVDEIGVGYVYDGGSVSRYILSEIKPLHNFLTQLQPFLKLKQKQANLVLKIIEQLPSAKESPDKFLEVCTWVDQIAALNDSKTRKTTSETVRAVLDSLPGSVGGLSPSQASSAASSASSSPGSGISEALRAGAGSGTGYNKEFLLYLAGFVDGDGSIYARIGPGQTYKFKHQLKLTFSVSQKTQRRWFLDKLVDEIGVGYVEDFGSVSKYILSQIKPLHNFLTQLQPFLKLKQKQANLVLKIIEQLPSAKESPDKFLEVCTWVDQIAALNDSKTRKTTSETVRAVLDSLSEKKKSSP

SEQ ID NO: 18 - protein, 354 aa, Artificial Sequence
  Synthesized
MNTKYNKEFLLYLAGFVDGDGSIHATIVPSQQYKFKHRLHLFFGVYQKTQRRWFLDKLVDEIGAGYVYDGGSVSRYILSQIKPLHNFLTQLQPFLKLKQKQANLVLKIIEQLPSAKESPDKFLEVCTWVDQIAALNDSKTRKTTSETVRAVLDSLPGSVGGLSPSQASSAASSASSSPGSGISEALRAGAGSGTGYNKEFLLYLAGFVDGDGSIYARIGPGQTYKFKHQLKLTFSVSQKTQRRWFLDKLVDEIGVGYVEDFGSVSKYILSQIKPLHNFLTQLQPFLKLKQKQANLVLKIIEQLPSAKESPDKFLEVCTWVDQIAALNDSKTRKTTSETVRAVLDSLSEKKKSSP

SEQ ID NO: 19 - protein, 354 aa, Artificial Sequence
  Synthesized
MNTKYNKEFLLYLAGFVDGDGSIHATIVPSQQYKFKHRLHLFFGVYQKTQRRWFLDKLVDEIGVGYVYDGGSVSRYILSQIKPLHNFLTQLQPFLKLKQKQANLVLKIIEQLPSAKESPDKFLEVCTWVDQIAALNDSKTRKTTSETVRAVLDSLPGSVGGLSPSQASSAASSASSSPGSGISEALRAGAGSGTGYNKEFLLYLAGFVDGDGSIYARILPVQVAKFKHQLRLTFRVGQKTQRRWFLDKLVDEIGVGYVSDSGSVSNYELSKIKPLHNFLTQLQPFLKLKQKQANLVLKIIEQLPSAKESPDKFLEVCTWVDQIAALNDSKTRKTTSETVRAVLDSLSEKKKSSP

SEQ ID NO: 20 - protein, 354 aa, Artificial Sequence
  Synthesized
MNTKYNKEFLLYLAGFVDGDGSICAGIQPSQYRKFKHGLWLGFYVVQKTQRRWFLDKLVDEIGVGYVYDRGSVSAYRLSQIKPLHNFLTQLQPFLKLKQKQANLVLKIIEQLPSAKESPDKFLEVCTWVDQIAALNDSKTRKTTSETVRAVLDSLPGSVGGLSPSQASSAASSASSSPGSGISEALRAGAGSGTGYNKEFLLYLAGFVDGDGSIFASIKPRQNAKFKHKLELCFTVGQKTQRRWFLDKLVDEIGVGYVADLGSVSEYRLSKIKPLHNFLTQLQPFLKLKQKQANLVLKIIEQLPSAKESPDKFLEVCTWVDQIAALNDSKTRKTTSETVRAVLDSLSEKKKSSP

SEQ ID NO: 21 - protein, 354 aa, Artificial Sequence
  Synthesized
MNTKYNKEFLLYLAGFVDGDGSIYATIRPDQVRKFKHQLTLYFRVSQKTQRRWFLDKLVDEIGVGYVNDCGSVSHYSLSQIKPLHNFLTQLQPFLKLKQKQANLVLKIIEQLPSAKESPDKFLEVCTWVDQIAALNDSKTRKTTSETVRAVLDSLPGSVGGLSPSQASSAASSASSSPGSGISEALRAGAGSGTGYNKEFLLYLAGFVDGDGSIYATIEPSQGYKFKHRLMLRFVVTQKTQRRWFLDKLVDEIGVGYVHDWGSVSSYRLSEIKPLHNFLTQLQPFLKLKQKQANLVLKIIEQLPSAKESPDKFLEVCTWVDQIAALNDSKTRKTTSETVRAVLDSLSEKKKSSP

SEQ ID NO: 22 - protein, 354 aa, Artificial Sequence
  Synthesized
MNTKYNKEFLLYLAGFVDGDGSIYASIYPRQAAKFKHALQLGFDVTQKTQRRWFLDKLVDEIGVGHVYDRGSVSSYRLSEIKPLHNFLTQLQPFLKLKQKQANLVLKIIEQLPSAKESPDKFLEVCTWVDQIAALNDSKTRKTTSETVRAVLDSLPGSVGGLSPSQASSAASSASSSPGSGISEALRAGAGSGTGYNKEFLLYLAGFVDGDGSIFARIRPRQSSKFKHRLTLAFTVGQKTQRRWFLDKLVDEIGVGYVADLGSVSEYRLSKIKPLHNFLTQLQPFLKLKQKQANLVLKIIEQLPSAKESPDKFLEVCTWVDQIAALNDSKTRKTTSETVRAVLDSLSEKKKSSP

SEQ ID NO: 23 - protein, 354 aa, Artificial Sequence
  Synthesized
MNTKYNKEFLLYLAGFVDGDGSIYATITPSQNSKFKHKLSLVFNVSQKTQRRWFLDKLVDEIGVGYVRDRGSVSDYRLSEIKPLHNFLTQLQPFLKLKQKQANLVLKIIEQLPSAKESPDKFLEVCTWVDQIAALNDSKTRKTTSETVRAVLDSLPGSVGGLSPSQASSAASSASSSPGSGISEALRAGAGSGTGYNKEFLLYLAGFVDGDGSIFARIRPGQRTKFKHKLALHFTVGQKTQRRWFLDKLVDEIGVGYVADLGSVSEYRLSQIKPLHNFLTQLQPFLKLKQKQANLVLKIIEQLPSAKESPDKFLEVCTWVDQIAALNDSKTRKTTSETVRAVLDSLSEKKKSSP

SEQ ID NO: 24 - protein, 354 aa, Artificial Sequence
  Synthesized
MNTKYNKEFLLYLAGFVDGDGSIYATIQPRQESKFKHSLRLYFDVTQKTQRRWFLDKLVDEIGVGYVYDSGSVSKYLLSQIKPLHNFLTQLQPFLKLKQKQANLVLKIIEQLPSAKESPDKFLEVCTWVDQIAALNDSKTRKTTSETVRAVLDSLPGSVGGLSPSQASSAASSASSSPGSGISEALRAGAGSGTGYNKEFLLYLAGFVDGDGSIHARIKPTQQVKFKHVLELRFSVYQKTQRRWFLDKLVDEIGVGYVTDSGGVSFYTLSKIKPLHNFLTQLQPFLKLKQKQANLVLKIIEQLPSAKESPDKFLEVCTWVDQIAALNDSKTRKTTSETVRAVLDSLSEKKKSSP

SEQ ID NO: 25 - protein, 354 aa, Artificial Sequence
  Synthesized
MNTKYNKEFLLYLAGFVDGDGSIFATIEPRQQAKFKHRLRLWFDVTQKTQRRWFLDKLVDEIGVGYVYDSGSVSKYVLSEIKPLHNFLTQLQPFLKLKQKQANLVLKIIEQLPSAKESPDKFLEVCTWVDQIAALNDSKTRKTTSETVRAVLDSLPGSVGGLSPSQASSAASSASSSPGSGISEALRAGAGSGTGYNKEFLLYLAGFVDGDGSIYARIKPTQQTKFKHSLELRFTVTQKTQRRWFLDKLVDEIGVGYVVDDGSVSFYTLSKIKPLHNFLTQLQPFLKLKQKQANLVLKIIEQLPSAKESPDKFLEVCTWVDQIAALNDSKTRKTTSETVRAVLDSLSEKKKSSP

SEQ ID NO: 26 - protein, 354 aa, Artificial Sequence
  Synthesized
MNTKYNKEFLLYLAGFVDGDGSIYATIEPRQQAKFKHRLRLWFDVTQKTQRRWFLDKLVDEIGVGYVYDLGSVSRYSLSEIKPLHNFLTQLQPFLKLKQKQANLVLKIIEQLPSAKESPDKFLEVCTWVDQIAALNDSKTRKTTSETVRAVLDSLPGSVGGLSPSQASSAASSASSSPGSGISEALRAGAGSGTGYNKEFLLYLAGFVDGDGSIFARIRPIQVSKFKHNLSLHFTVHQKTQRRWFLDKLVDEIGVGYVVDDGSVSTYTLSQIKPLHNFLTQLQPFLKLKQKQANLVLKIIEQLPSAKESPDKFLEVCTWVDQIAALNDSKTRKTTSETVRAVLDSLSEKKKSSP

SEQ ID NO: 27 - protein, 354 aa, Artificial Sequence
  Synthesized
MNTKYNKEFLLYLAGFVDGDGSIYATIQPRQESKFKHSLRLYFDVTQKTQRRWFLDKLVDEIGVGYVYDSGSVSKYLLSQIKPLHNFLTQLQPFLKLKQKQANLVLKIIEQLPSAKESPDKFLEVCTWVDQIAALNDSKTRKTTSETVRAVLDSLPGSVGGLSPSQASSAASSASSSPGSGISEALRAGAGSGTGYNKEFLLYLAGFVDGDGSIFARIKPCQQVKFKHTLSLHFTVFQKTQRRWFLDKLVDEIGVGYVCDSGSVSSYVLSKIKPLHNFLTQLQPFLKLKQKQANLVLKIIEQLPSAKESPDKFLEVCTWVDQIAALNDSKTRKTTSETVRAVLDSLSEKKKSSP

SEQ ID NO: 28 - protein, 147 aa, Artificial Sequence
  Synthesized
KEFLLYLAGFVDGDGSIYATINPVQWNKFKHQLRLTFAVTQKTQRRWFLDKLVDEIGVGYVSDWGSVSQYKLSEIKPLHNFLTQLQPFLKLKQKQANLVLKIIEQLPSAKESPDKFLEVCTWVDQIAALNDSKTRKTTSETVRAVLD

SEQ ID NO: 29 - protein, 147 aa, Artificial Sequence
  Synthesized
KEFLLYLAGFVDGDGSIFATIDPEQTGKFKHKLRLRFVVTQKTQRRWFLDKLVDEIGVGYVTDWGSVSYYRLSEIKPLHNFLTQLQPFLKLKQKQANLVLKIIEQLPSAKESPDKFLEVCTWVDQIAALNDSKTRKTTSETVRAVLD

SEQ ID NO: 30 - protein, 147 aa, Artificial Sequence
  Synthesized
KEFLLYLAGFVDGDGSIFASIEPIQYSKFKHRLKLYFAVSQKTQRRWFLDKLVDEIGVGYVTDHGSVSTYRLSKIKPLHNFLTQLQPFLKLKQKQANLVLKIIEQLPSAKESPDKFLEVCTWVDQIAALNDSKTRKTTSETVRAVLD

SEQ ID NO: 31 - protein, 147 aa, Artificial Sequence
  Synthesized
KEFLLYLAGFVDGDGSIYAAIEPTQCAKFKHKLRLLFAVTQKTQRRWFLDKLVDEIGVGYVYDQGSVSTYRLSQIKPLHNFLTQLQPFLKLKQKQANLVLKIIEQLPSAKESPDKFLEVCTWVDQIAALNDSKTRKTTSETVRAVLD

SEQ ID NO: 32 - protein, 147 aa, Artificial Sequence
  Synthesized
KEFLLYLAGFVDGDGSIFATIQPSQHRKFKHQLVLWFRVTQKTQRRWFLDKLVDEIGVGYVRDTGSVSYYSLSQIKPLHNFLTQLQPFLKLKQKQANLVLKIIEQLPSAKESPDKFLEVCTWVDQIAALNDSKTRKTTSETVRAVLD

SEQ ID NO: 33 - protein, 147 aa, Artificial Sequence
  Synthesized
KEFLLYLAGFVDGDGSIYATIRPDQVRKFKHQLTLYFRVSQKTQRRWFLDKLVDEIGVGYVNDCGSVSHYSLSQIKPLHNFLTQLQPFLKLKQKQANLVLKIIEQLPSAKESPDKFLEVCTWVDQIAALNDSKTRKTTSETVRAVLD

SEQ ID NO: 34 - protein, 147 aa, Artificial Sequence
  Synthesized
KEFLLYLAGFVDGDGSIFATIQPSQHRKFKHQLVLWFRVTQKTQRRWFLDKLVDEIGVGYVRDTGSVSYYSLSKIKPLHNFLTQLQPFLKLKQKQANLVLKIIEQLPSAKESPDKFLEVCTWVDQIAALNDSKTRKTTSETVRAVLD

SEQ ID NO: 35 - protein, 147 aa, Artificial Sequence
  Synthesized
KEFLLYLAGFVDGDGSIYATIQPGQTRKFKHQLSLWFRVTQKTQRRWFLDKLVDEIGVGYVSDAGSVSHYSLSQIKPLHNFLTQLQPFLKLKQKQANLVLKIIEQLPSAKESPDKFLEVCTWVDQIAALNDSKTRKTTSETVRAVLD

SEQ ID NO: 36 - protein, 147 aa, Artificial Sequence
  Synthesized
KEFLLYLAGFVDGDGSIHATIVPSQQYKFKHRLHLFFGVYQKTQRRWFLDKLVDEIGVGYVYDGGSVSRYILSEIKPLHNFLTQLQPFLKLKQKQANLVLKIIEQLPSAKESPDKFLEVCTWVDQIAALNDSKTRKTTSETVRAVLD

SEQ ID NO: 37 - protein, 147 aa, Artificial Sequence; identical to SEQ ID NO: 36
  Synthesized

SEQ ID NO: 38 - protein, 147 aa, Artificial Sequence
  Synthesized
KEFLLYLAGFVDGDGSIHATIVPSQQYKFKHRLHLFFGVYQKTQRRWFLDKLVDEIGAGYVYDGGSVSRYILSQIKPLHNFLTQLQPFLKLKQKQANLVLKIIEQLPSAKESPDKFLEVCTWVDQIAALNDSKTRKTTSETVRAVLD

SEQ ID NO: 39 - protein, 147 aa, Artificial Sequence
  Synthesized
KEFLLYLAGFVDGDGSIHATIVPSQQYKFKHRLHLFFGVYQKTQRRWFLDKLVDEIGVGYVYDGGSVSRYILSQIKPLHNFLTQLQPFLKLKQKQANLVLKIIEQLPSAKESPDKFLEVCTWVDQIAALNDSKTRKTTSETVRAVLD

SEQ ID NO: 40 - protein, 147 aa, Artificial Sequence
  Synthesized
KEFLLYLAGFVDGDGSIYARILPVQVAKFKHQLRLTFRVGQKTQRRWFLDKLVDEIGVGYVSDSGSVSNYELSQIKPLHNFLTQLQPFLKLKQKQANLVLKIIEQLPSAKESPDKFLEVCTWVDQIAALNDSKTRKTTSETVRAVLD

SEQ ID NO: 41 - protein, 147 aa, Artificial Sequence
  Synthesized
KEFLLYLAGFVDGDGSIYARIGPGQTYKFKHQLKLTFSVSQKTQRRWFLDKLVDEIGVGYVEDFGSVSKYILSQIKPLHNFLTQLQPFLKLKQKQANLVLKIIEQLPSAKESPDKFLEVCTWVDQIAALNDSKTRKTTSETVRAVLD

SEQ ID NO: 42 - protein, 147 aa, Artificial Sequence; identical to SEQ ID NO: 41
  Synthesized

SEQ ID NO: 43 - protein, 147 aa, Artificial Sequence
  Synthesized
KEFLLYLAGFVDGDGSIYARILPVQVAKFKHQLRLTFRVGQKTQRRWFLDKLVDEIGVGYVSDSGSVSNYELSKIKPLHNFLTQLQPFLKLKQKQANLVLKIIEQLPSAKESPDKFLEVCTWVDQIAALNDSKTRKTTSETVRAVLD

SEQ ID NO: 44 - protein, 147 aa, Artificial Sequence
  Synthesized
KEFLLYLAGFVDGDGSICAGIQPSQYRKFKHGLWLGFYVVQKTQRRWFLDKLVDEIGVGYVYDRGSVSAYRLSQIKPLHNFLTQLQPFLKLKQKQANLVLKIIEQLPSAKESPDKFLEVCTWVDQIAALNDSKTRKTTSETVRAVLD

SEQ ID NO: 45 - protein, 147 aa, Artificial Sequence; identical to SEQ ID NO: 33
  Synthesized

SEQ ID NO: 46 - protein, 147 aa, Artificial Sequence
  Synthesized
KEFLLYLAGFVDGDGSIYASIYPRQAAKFKHALQLGFDVTQKTQRRWFLDKLVDEIGVGHVYDRGSVSSYRLSEIKPLHNFLTQLQPFLKLKQKQANLVLKIIEQLPSAKESPDKFLEVCTWVDQIAALNDSKTRKTTSETVRAVLD

SEQ ID NO: 47 - protein, 147 aa, Artificial Sequence
  Synthesized
KEFLLYLAGFVDGDGSIYATITPSQNSKFKHKLSLVFNVSQKTQRRWFLDKLVDEIGVGYVRDRGSVSDYRLSEIKPLHNFLTQLQPFLKLKQKQANLVLKIIEQLPSAKESPDKFLEVCTWVDQIAALNDSKTRKTTSETVRAVLD

SEQ ID NO: 48 - protein, 147 aa, Artificial Sequence
  Synthesized
KEFLLYLAGFVDGDGSIFASIKPRQNAKFKHKLELCFTVGQKTQRRWFLDKLVDEIGVGYVADLGSVSEYRLSKIKPLHNFLTQLQPFLKLKQKQANLVLKIIEQLPSAKESPDKFLEVCTWVDQIAALNDSKTRKTTSETVRAVLD

SEQ ID NO: 49 - protein, 147 aa, Artificial Sequence
  Synthesized
KEFLLYLAGFVDGDGSIYATIEPSQGYKFKHRLMLRFVVTQKTQRRWFLDKLVDEIGVGYVHDWGSVSSYRLSEIKPLHNFLTQLQPFLKLKQKQANLVLKIIEQLPSAKESPDKFLEVCTWVDQIAALNDSKTRKTTSETVRAVLD

SEQ ID NO: 50 - protein, 147 aa, Artificial Sequence
  Synthesized
KEFLLYLAGFVDGDGSIFARIRPRQSSKFKHRLTLAFTVGQKTQRRWFLDKLVDEIGVGYVADLGSVSEYRLSKIKPLHNFLTQLQPFLKLKQKQANLVLKIIEQLPSAKESPDKFLEVCTWVDQIAALNDSKTRKTTSETVRAVLD

SEQ ID NO: 51 - protein, 147 aa, Artificial Sequence
  Synthesized
KEFLLYLAGFVDGDGSIFARIRPGQRTKFKHKLALHFTVGQKTQRRWFLDKLVDEIGVGYVADLGSVSEYRLSQIKPLHNFLTQLQPFLKLKQKQANLVLKIIEQLPSAKESPDKFLEVCTWVDQIAALNDSKTRKTTSETVRAVLD

SEQ ID NO: 52 - protein, 147 aa, Artificial Sequence
  Synthesized
KEFLLYLAGFVDGDGSIYATIQPRQESKFKHSLRLYFDVTQKTQRRWFLDKLVDEIGVGYVYDSGSVSKYLLSQIKPLHNFLTQLQPFLKLKQKQANLVLKIIEQLPSAKESPDKFLEVCTWVDQIAALNDSKTRKTTSETVRAVLD

SEQ ID NO: 53 - protein, 147 aa, Artificial Sequence
  Synthesized
KEFLLYLAGFVDGDGSIFATIEPRQQAKFKHRLRLWFDVTQKTQRRWFLDKLVDEIGVGYVYDSGSVSKYVLSEIKPLHNFLTQLQPFLKLKQKQANLVLKIIEQLPSAKESPDKFLEVCTWVDQIAALNDSKTRKTTSETVRAVLD

SEQ ID NO: 54 - protein, 147 aa, Artificial Sequence
  Synthesized
KEFLLYLAGFVDGDGSIYATIEPRQQAKFKHRLRLWFDVTQKTQRRWFLDKLVDEIGVGYVYDLGSVSRYSLSEIKPLHNFLTQLQPFLKLKQKQANLVLKIIEQLPSAKESPDKFLEVCTWVDQIAALNDSKTRKTTSETVRAVLD

SEQ ID NO: 55 - protein, 147 aa, Artificial Sequence; identical to SEQ ID NO: 52
  Synthesized

SEQ ID NO: 56 - protein, 147 aa, Artificial Sequence
  Synthesized
KEFLLYLAGFVDGDGSIHARIKPTQQVKFKHVLELRFSVYQKTQRRWFLDKLVDEIGVGYVTDSGGVSFYTLSKIKPLHNFLTQLQPFLKLKQKQANLVLKIIEQLPSAKESPDKFLEVCTWVDQIAALNDSKTRKTTSETVRAVLD

SEQ ID NO: 57 - protein, 147 aa, Artificial Sequence
  Synthesized
KEFLLYLAGFVDGDGSIYARIKPTQQTKFKHSLELRFTVTQKTQRRWFLDKLVDEIGVGYVVDDGSVSFYTLSKIKPLHNFLTQLQPFLKLKQKQANLVLKIIEQLPSAKESPDKFLEVCTWVDQIAALNDSKTRKTTSETVRAVLD

SEQ ID NO: 58 - protein, 147 aa, Artificial Sequence
  Synthesized
KEFLLYLAGFVDGDGSIFARIRPIQVSKFKHNLSLHFTVHQKTQRRWFLDKLVDEIGVGYVVDDGSVSTYTLSQIKPLHNFLTQLQPFLKLKQKQANLVLKIIEQLPSAKESPDKFLEVCTWVDQIAALNDSKTRKTTSETVRAVLD

SEQ ID NO: 59 - protein, 147 aa, Artificial Sequence
  Synthesized
KEFLLYLAGFVDGDGSIFARIKPCQQVKFKHTLSLHFTVFQKTQRRWFLDKLVDEIGVGYVCDSGSVSSYVLSKIKPLHNFLTQLQPFLKLKQKQANLVLKIIEQLPSAKESPDKFLEVCTWVDQIAALNDSKTRKTTSETVRAVLD

SEQ ID NO: 60 - DNA, 2847 bp, Artificial Sequence
  Synthesized
tagcactctatcacggccatattctggcagggtcagtggctccaactaacatttgtttggtactttacagtttattaaatagatgtttatatggagaagctctcatttctttctcagaagagcctggctaggaaggtggatgaggcaccatattcattttgcaggtgaaattcctgagatgtaaggagctgctgtgacttgctcaaggccttatatcaagtaaacggtagcgctggggcttagacgcaggtgttctgatttatagttcaaaacctctatcaatgagagagcaatctcctggtaatgtgatagatttcccaacttaatgccaacataccataaacctcccattctgctaatgcccagcctaagttggggagaccactccagattccaagatgtacagtttgctttgctgggcctttttcccatgcctgcctttactctgccagagttatattgctggggttttgaagaagatcctattaaataaaagaataagcagtattattaagtagccctgcatttcaggtttccttgagtggcaggccaggcctggccgtgaacgttcactgaaatcatggcctcttggccaagattgatagcttgtgccttgtcgagacagagaagactcttgcgtttctgataggcacctattggtcttactgacatccactttgcctttctctccacaggcggcggtggcgagggcagaggaagtcttctaacatgcggtgacgtggaggagaatcccggccctatggcgctcccagtgacagccttacttttacctctggcgttattattgcacgcggctcgtcctgacatacagatgactcagactacctcttccctatctgcttctttaggcgaccgagtaacaatatcttgccgggccagccaggacatctcaaaatacttaaactggtatcagcagaagccggacggaacagttaagttgctcatttaccacacgtcgagattacactcaggcgttcctagccgattttcgggttccggttccggtacggactacagcctgacaatcagtaaccttgagcaggaggacatcgccacctacttctgtcagcagggcaacacgctcccgtacacattcggtgggggaactaagctggagattaccggaggcggtggcagcggtggcggcggcagcgggggtggcggctcggaggtcaagttacaggagagcggaccgggcttggtcgcacctagccagagcctctcagtcacgtgcactgtgtctggagtcagtctcccagactacggggtatcatggatacgacagccgcctagaaagggcttagagtggctgggggttatctggggaagtgaaaccacatactacaactcagctctcaagagccgcctcaccatcattaaggacaacagtaagtcgcaggttttcttaaagatgaactctctccagactgacgacaccgctatttactactgcgcgaagcactactactacggcgggagttacgcaatggactactggggtcagggcacttctgtgaccgtatccagcactactaccccagccccacgtccccccacgccagctccaacgatagcaagtcagcccttatctcttcgccctgaggcttgcaggcccgcggcgggcggcgccgttcacacgcgaggactagacttcgcctgcgacatctacatctgggcaccactagccgggacttgcggagtgttgttgttgagcttggtaataacgctctactgcaaagcgagccgcaaaaaagcggcggcggcggcgaaaagcccgtttgcgagcccggcgagcagcgcgcaggaagaagatgcgagcagctgccgcgcgccgagcgaagaagaaggcagctgcgaactgagagtgaagttctctcgctccgcggacgcacccgcttaccagcagggtcagaaccagctatacaacgagttaaacctggggcgccgggaggagtacgacgtgttagacaagcgtagaggtagggacccggagatgggaggcaagcctcggagaaagaacccccaggagggcctgtacaacgaactccagaaggacaagatggctgaggcgtactcggagattggtatgaagggcgagagacgtcgcggaaagggacacgacggcttataccaggggctttccaccgcgaccaaggacacatacgacgcgctgcacatgcaagccttaccacctcgatgaggtaccagcggccgcgatccagacatgataagatacattgatgagtttggacaaaccacaactagaatgcagtgaaaaaaatgctttatttgtgaaatttgtgatgctattgctttatttgtaaccattataagctgcaataaacaagttaacaacaacaattgcattcattttatgtttcaggttcagggggaggtgtgggaggttttttaaagcaagtaagtgcctgtccctgagtcccagtccatcacgagcagctggtttctaagatgctatttcccgtataaagcatgagaccgtgacttgccagccccacagagccccgcccttgtccatcactggcatctggactccagcctgggttggggcaaagagggaaatgagatcatgtcctaaccctgatcctcttgtcccacagatatccagaaccctgaccctgccgtgtaccagctgagagactctaaatccagtgacaagtctgtctgcctattcaccgattttgattctcaaacaaatgtgtcacaaagtaaggattctgatgtgtatatcacagacaaaactgtgctagacatgaggtctatggacttcaagagcaacagtgctgtggcctggagcaacaaatctga

SEQ ID NO: 61 - DNA, 2847 bp, Artificial Sequence
  Synthesized
catgctaatcctccggcaaacctctgtttcctcctcaaaaggcaggaggtcggaaagaataaacaatgagagtcacattaaaaacacaaaatcctacggaaatactgaagaatgagtctcagcactaaggaaaagcctccagcagctcctgctttctgagggtgaaggatagacgctgtggctctgcatgactcactagcactctatcacggccatattctggcagggtcagtggctccaactaacatttgtttggtactttacagtttattaaatagatgtttatatggagaagctctcatttctttctcagaagagcctggctaggaaggtggatgaggcaccatattcattttgcaggtgaaattcctgagatgtaaggagctgctgtgacttgctcaaggccttatatcaagtaaacggtagcgctggggcttagacgcaggtgttctgatttatagttcaaaacctctatcaatgagagagcaatctcctggtaatgtgatagatttcccaacttaatgccaacataccataaacctcccattctgctaatgcccagcctaagttggggagaccactccagattccaagatgtacagtttgctttgccttgtcgagacagagaagactcttgcgtttctgataggcacctattggtcttactgacatccactttgcctttctctccacaggcggcagcggcgagggcagaggaagtcttctaacatgcggtgacgtggaggagaatcccggccctatggcgctcccagtgacagccttacttttacctctggcgttattattgcacgcggctcgtcctgacatacagatgactcagactacctcttccctatctgcttctttaggcgaccgagtaacaatatcttgccgggccagccaggacatctcaaaatacttaaactggtatcagcagaagccggacggaacagttaagttgctcatttaccacacgtcgagattacactcaggcgttcctagccgattttcgggttccggttccggtacggactacagcctgacaatcagtaaccttgagcaggaggacatcgccacctacttctgtcagcagggcaacacgctcccgtacacattcggtgggggaactaagctggagattaccggaggcggtggcagcggtggcggcggcagcgggggtggcggctcggaggtcaagttacaggagagcggaccgggcttggtcgcacctagccagagcctctcagtcacgtgcactgtgtctggagtcagtctcccagactacggggtatcatggatacgacagccgcctagaaagggcttagagtggctgggggttatctggggaagtgaaaccacatactacaactcagctctcaagagccgcctcaccatcattaaggacaacagtaagtcgcaggttttcttaaagatgaactctctccagactgacgacaccgctatttactactgcgcgaagcactactactacggcgggagttacgcaatggactactggggtcagggcacttctgtgaccgtatccagcactactaccccagccccacgtccccccacgccagctccaacgatagcaagtcagcccttatctcttcgccctgaggcttgcaggcccgcggcgggcggcgccgttcacacgcgaggactagacttcgcctgcgacatctacatctgggcaccactagccgggacttgcggagtgttgttgttgagcttggtaataacgctctactgcaaagcgagccgcaaaaaagcggcggcggcggcgaaaagcccgtttgcgagcccggcgagcagcgcgcaggaagaagatgcgagcagctgccgcgcgccgagcgaagaagaaggcagctgcgaactgagagtgaagttctctcgctccgcggacgcacccgcttaccagcagggtcagaaccagctatacaacgagttaaacctggggcgccgggaggagtacgacgtgttagacaagcgtagaggtagggacccggagatgggaggcaagcctcggagaaagaacccccaggagggcctgtacaacgaactccagaaggacaagatggctgaggcgtactcggagattggtatgaagggcgagagacgtcgcggaaagggacacgacggcttataccaggggctttccaccgcgaccaaggacacatacgacgcgctgcacatgcaagccttaccacctcgatgaggtaccagcggccgcgatccagacatgataagatacattgatgagtttggacaaaccacaactagaatgcagtgaaaaaaatgctttatttgtgaaatttgtgatgctattgctttatttgtaaccattataagctgcaataaacaagttaacaacaacaattgcattcattttatgtttcaggttcagggggaggtgtgggaggttttttaaagcaagtaattgctgggcctttttcccatgcctgcctttactctgccagagttatattgctggggttttgaagaagatcctattaaataaaagaataagcagtattattaagtagccctgcatttcaggtttccttgagtggcaggccaggcctggccgtgaacgttcactgaaatcatggcctcttggccaagattgatagcttgtgcctgtccctgagtcccagtccatcacgagcagctggtttctaagatgctatttcccgtataaagcatgagaccgtgacttgccagccccacagagccccgcccttgtccatcactggcatctggactccagcctgggttggggcaaagagggaaatgagatcatgtcctaaccctgatcctcttgtcccacagatatccagaacc

SEQ ID NO: 62 - DNA, 2229 bp, Artificial Sequence
  Synthesized
catgctaatcctccggcaaacctctgtttcctcctcaaaaggcaggaggtcggaaagaataaacaatgagagtcacattaaaaacacaaaatcctacggaaatactgaagaatgagtctcagcactaaggaaaagcctccagcagctcctgctttctgagggtgaaggatagacgctgtggctctgcatgactcactagcactctatcacggccatattctggcagggtcagtggctccaactaacatttgtttggtactttacagtttattaaatagatgtttatatggagaagctctcatttctttctcagaagagcctggctaggaaggtggatgaggcaccatattcattttgcaggtgaaattcctgagatgtaaggagctgctgtgacttgccttgtcgagacagagaagactcttgcgtttctgataggcacctattggtcttactgacatccactttgcctttctctccacaggcggcggtggcgagggcagaggaagtcttctaacatgcggtgacgtggaggagaatcccggccctatggcgctcccagtgacagccttacttttacctctggcgttattattgcacgcggctcgtcctgacatacagatgactcagactacctcttccctatctgcttctttaggcgaccgagtaacaatatcttgccgggccagccaggacatctcaaaatacttaaactggtatcagcagaagccggacggaacagttaagttgctcatttaccacacgtcgagattacactcaggcgttcctagccgattttcgggttccggttccggtacggactacagcctgacaatcagtaaccttgagcaggaggacatcgccacctacttctgtcagcagggcaacacgctcccgtacacattcggtgggggaactaagctggagattaccggaggcggtggcagcggtggcggcggcagcgggggtggcggctcggaggtcaagttacaggagagcggaccgggcttggtcgcacctagccagagcctctcagtcacgtgcactgtgtctggagtcagtctcccagactacggggtatcatggatacgacagccgcctagaaagggcttagagtggctgggggttatctggggaagtgaaaccacatactacaactcagctctcaagagccgcctcaccatcattaaggacaacagtaagtcgcaggttttcttaaagatgaactctctccagactgacgacaccgctatttactactgcgcgaagcactactactacggcgggagttacgcaatggactactggggtcagggcacttctgtgaccgtatccagcactactaccccagccccacgtccccccacgccagctccaacgatagcaagtcagcccttatctcttcgccctgaggcttgcaggcccgcggcgggcggcgccgttcacacgcgaggactagacttcgcctgcgacatctacatctgggcaccactagccgggacttgcggagtgttgttgttgagcttggtaataacgctctactgcaaagcgagccgcaaaaaagcggcggcggcggcgaaaagcccgtttgcgagcccggcgagcagcgcgcaggaagaagatgcgagcagctgccgcgcgccgagcgaagaagaaggcagctgcgaactgagagtgaagttctctcgctccgcggacgcacccgcttaccagcagggtcagaaccagctatacaacgagttaaacctggggcgccgggaggagtacgacgtgttagacaagcgtagaggtagggacccggagatgggaggcaagcctcggagaaagaacccccaggagggcctgtacaacgaactccagaaggacaagatggctgaggcgtactcggagattggtatgaagggcgagagacgtcgcggaaagggacacgacggcttataccaggggctttccaccgcgaccaaggacacatacgacgcgctgcacatgcaagccttaccacctcgatgaggtaccagcggccgcgatccagacatgataagatacattgatgagtttggacaaaccacaactagaatgcagtgaaaaaaatgctttatttgtgaaatttgtgatgctattgctttatttgtaaccattataagctgcaataaacaagttaacaacaacaattgcattcattttatgtttcaggttcagggggaggtgtgggaggttttttaaagcaagtaa

SEQ ID NO: 63 - DNA, 2524 bp, Artificial Sequence
  Synthesized
gttggccactccctctctgcgcgctcgctcgctcactgaggccgggcgaccaaaggtcgcccgacgcccgggctttgcccgggcggcctcagtgagcgagcgagcgcgcagagagggagtggccaactccatcactaggggttcctacgcgtccagcagctcctgctttctgagggtgaaggatagacgctgtggctctgcatgactcactagcactctatcacggccatattctggcagggtcagtggctccaactaacatttgtttggtactttacagtttattaaatagatgtttatatggagaagctctcatttctttctcagaagagcctggctaggaaggtggatgaggcaccatattcattttgcaggtgaaattcctgagatgtaaggagctgctgtgacttgctcaaggccttatatcaagtaaacggtagcgctggggcttagacgcaggtgttctgatttatagttcaaaacctctatcaatgagagagcaatctcctggtaatgtgatagatttcccaacttaatgccaacataccataaacctcccattctgctaatgcccagcctaagttggggagaccactccagattccaagatgtacagtttgctttgctgggcctttttcccatgcctgcctttactctgccagagttatattgctggggttttgaagaagatcctattaaataaaagaataagcagtattattaagtagccctgcatttcaggtttccttgagtggcaggccaggcctggccgtgaacgttcactgaaatcatggcctcttggccaagattgatagcttgtgccttgtcgagacagagaagactcttgcgtttctgataggcacctattggtcttactgacatccactttgcctttctctccacaggcggcggtggcgagggcagaggaagtcttctaacatgcggtgacgtggaggagaatcccggccccatggtgagcaagggcgaggagctgttcaccggggtggtgcccatcctggtcgagctggacggcgacgtaaacggccacaagttcagcgtgtccggcgagggcgagggcgatgccacctacggcaagctgaccctgaagttcatctgcaccaccggcaagctgcccgtgccctggcccaccctcgtgaccaccctgacctacggagtgcagtgcttcagccgctaccccgaccacatgaagcagcacgacttcttcaagtccgccatgcccgaaggctacgtccaggagcgcaccatcttcttcaaggacgacggcaactacaagacccgcgccgaggtgaagttcgagggcgacaccctggtgaaccgcatcgagctgaagggcatcgacttcaaggaggacggcaacatcctggggcacaagctggagtacaactacaacagccacaacgtctatatcatggccgacaagcagaagaacggcatcaaggtgaacttcaagatccgccacaacatcgaggacggcagcgtgcagctcgccgaccactaccagcagaacacccccatcggcgacggccccgtgctgctgcccgacaaccactacctgagcacccagtccgccctgagcaaagaccccaacgagaagcgcgatcacatggtcctgctggagttcgtgaccgccgccgggatcactctcggcatggacgagctgtacaagtaacctaggtaccgcggccgcgatccagacatgataagatacattgatgagtttggacaaaccacaactagaatgcagtgaaaaaaatgctttatttgtgaaatttgtgatgctattgctttatttgtaaccattataagctgcaataaacaagttaacaacaacaattgcattcattttatgtttcaggttcagggggaggtgtgggaggttttttaaagcaagtaagtgcctgtccctgagtcccagtccatcacgagcagctggtttctaagatgctatttcccgtataaagcatgagaccgtgacttgccagccccacagagccccgcccttgtccatcactggcatctggactccagcctgggttggggcaaagagggaaatgagatcatgtcctaaccctgatcctcttgtcccacagatatccagaaccctgaccctgccgtgtaccagctgagagactctaaatccagtgacaagtctgtctgcctattcaccgattttgattctcaaacaaatgtgtcacaaagtaaggattctgatgtgtatatcacagacaaaactgtgctagacatgaggtctatggacttcaagagcaacagtgctgtggcctggagcaacaaatctgactttgcatgtgcaaacgccttcaacaacagcattattccagaagacaccttcttccccagcccaggtaaggggaattgatggagttggccactccctctctgcgcgctcgctcgctcactgaggccgcccgggcaaagcccgggcgtcgggcgacctttggtcgcccggcctcagtgagcgagcgagcgcgcagagagggagtgg

SEQ ID NO: 64 - DNA, 3262 bp, Artificial Sequence
  Synthesized
gttggccactccctctctgcgcgctcgctcgctcactgaggccgggcgaccaaaggtcgcccgacgcccgggctttgcccgggcggcctcagtgagcgagcgagcgcgcagagagggagtggccaactccatcactaggggttcctacgcgtccagcagctcctgctttctgagggtgaaggatagacgctgtggctctgcatgactcactagcactctatcacggccatattctggcagggtcagtggctccaactaacatttgtttggtactttacagtttattaaatagatgtttatatggagaagctctcatttctttctcagaagagcctggctaggaaggtggatgaggcaccatattcattttgcaggtgaaattcctgagatgtaaggagctgctgtgacttgctcaaggccttatatcaagtaaacggtagcgctggggcttagacgcaggtgttctgatttatagttcaaaacctctatcaatgagagagcaatctcctggtaatgtgatagatttcccaacttaatgccaacataccataaacctcccattctgctaatgcccagcctaagttggggagaccactccagattccaagatgtacagtttgctttgctgggcctttttcccatgcctgcctttactctgccagagttatattgctggggttttgaagaagatcctattaaataaaagaataagcagtattattaagtagccctgcatttcaggtttccttgagtggcaggccaggcctggccgtgaacgttcactgaaatcatggcctcttggccaagattgatagcttgtgccttgtcgagacagagaagactcttgcgtttctgataggcacctattggtcttactgacatccactttgcctttctctccacaggcggcggtggcgagggcagaggaagtcttctaacatgcggtgacgtggaggagaatcccggccccatggcgctcccagtgacagccttacttttacctctggcgttattattgcacgcggctcgtcctgacatacagatgactcagactacctcttccctatctgcttctttaggcgaccgagtaacaatatcttgccgggccagccaggacatctcaaaatacttaaactggtatcagcagaagccggacggaacagttaagttgctcatttaccacacgtcgagattacactcaggcgttcctagccgattttcgggttccggttccggtacggactacagcctgacaatcagtaaccttgagcaggaggacatcgccacctacttctgtcagcagggcaacacgctcccgtacacattcggtgggggaactaagctggagattaccggaggcggtggcagcggtggcggcggcagcgggggtggcggctcggaggtcaagttacaggagagcggaccgggcttggtcgcacctagccagagcctctcagtcacgtgcactgtgtctggagtcagtctcccagactacggggtatcatggatacgacagccgcctagaaagggcttagagtggctgggggttatctggggaagtgaaaccacatactacaactcagctctcaagagccgcctcaccatcattaaggacaacagtaagtcgcaggttttcttaaagatgaactctctccagactgacgacaccgctatttactactgcgcgaagcactactactacggcgggagttacgcaatggactactggggtcagggcacttctgtgaccgtatccagcactactaccccagccccacgtccccccacgccagctccaacgatagcaagtcagcccttatctcttcgccctgaggcttgcaggcccgcggcgggcggcgccgttcacacgcgaggactagacttcgcctgcgacatctacatctgggcaccactagccgggacttgcggagtgttgttgttgagcttggtaataacgctctactgcaaagcgagccgcaaaaaagcggcggcggcggcgaaaagcccgtttgcgagcccggcgagcagcgcgcaggaagaagatgcgagcagctgccgcgcgccgagcgaagaagaaggcagctgcgaactgagagtgaagttctctcgctccgcggacgcacccgcttaccagcagggtcagaaccagctatacaacgagttaaacctggggcgccgggaggagtacgacgtgttagacaagcgtagaggtagggacccggagatgggaggcaagcctcggagaaagaacccccaggagggcctgtacaacgaactccagaaggacaagatggctgaggcgtactcggagattggtatgaagggcgagagacgtcgcggaaagggacacgacggcttataccaggggctttccaccgcgaccaaggacacatacgacgcgctgcacatgcaagccttaccacctcgatgaggtaccagcggccgcgatccagacatgataagatacattgatgagtttggacaaaccacaactagaatgcagtgaaaaaaatgctttatttgtgaaatttgtgatgctattgctttatttgtaaccattataagctgcaataaacaagttaacaacaacaattgcattcattttatgtttcaggttcagggggaggtgtgggaggttttttaaagcaagtaagtgcctgtccctgagtcccagtccatcacgagcagctggtttctaagatgctatttcccgtataaagcatgagaccgtgacttgccagccccacagagccccgcccttgtccatcactggcatctggactccagcctgggttggggcaaagagggaaatgagatcatgtcctaaccctgatcctcttgtcccacagatatccagaaccctgaccctgccgtgtaccagctgagagactctaaatccagtgacaagtctgtctgcctattcaccgattttgattctcaaacaaatgtgtcacaaagtaaggattctgatgtgtatatcacagacaaaactgtgctagacatgaggtctatggacttcaagagcaacagtgctgtggcctggagcaacaaatctgactttgcatgtgcaaacgccttcaacaacagcattattccagaagacaccttcttccccagcccaggtaaggggaattgatggagttggccactccctctctgcgcgctcgctcgctcactgaggccgcccgggcaaagcccgggcgtcgggcgacctttggtcgcccggcctcagtgagcgagcgagcgcgcagagagggagtgg

SEQ ID NO: 65 - DNA, 2524 bp, Artificial Sequence
  Synthesized
gttggccactccctctctgcgcgctcgctcgctcactgaggccgggcgaccaaaggtcgcccgacgcccgggctttgcccgggcggcctcagtgagcgagcgagcgcgcagagagggagtggccaactccatcactaggggttcctacgcgtccagcagctcctgctttctgagggtgaaggatagacgctgtggctctgcatgactcactagcactctatcacggccatattctggcagggtcagtggctccaactaacatttgtttggtactttacagtttattaaatagatgtttatatggagaagctctcatttctttctcagaagagcctggctaggaaggtggatgaggcaccatattcattttgcaggtgaaattcctgagatgtaaggagctgctgtgacttgctcaaggccttatatcaagtaaacggtagcgctggggcttagacgcaggtgttctgatttatagttcaaaacctctatcaatgagagagcaatctcctggtaatgtgatagatttcccaacttaatgccaacataccataaacctcccattctgctaatgcccagcctaagttggggagaccactccagattccaagatgtacagtttgctttgccttgtcgagacagagaagactcttgcgtttctgataggcacctattggtcttactgacatccactttgcctttctctccacaggcggcggtggcgagggcagaggaagtcttctaacatgcggtgacgtggaggagaatcccggccccatggtgagcaagggcgaggagctgttcaccggggtggtgcccatcctggtcgagctggacggcgacgtaaacggccacaagttcagcgtgtccggcgagggcgagggcgatgccacctacggcaagctgaccctgaagttcatctgcaccaccggcaagctgcccgtgccctggcccaccctcgtgaccaccctgacctacggagtgcagtgcttcagccgctaccccgaccacatgaagcagcacgacttcttcaagtccgccatgcccgaaggctacgtccaggagcgcaccatcttcttcaaggacgacggcaactacaagacccgcgccgaggtgaagttcgagggcgacaccctggtgaaccgcatcgagctgaagggcatcgacttcaaggaggacggcaacatcctggggcacaagctggagtacaactacaacagccacaacgtctatatcatggccgacaagcagaagaacggcatcaaggtgaacttcaagatccgccacaacatcgaggacggcagcgtgcagctcgccgaccactaccagcagaacacccccatcggcgacggccccgtgctgctgcccgacaaccactacctgagcacccagtccgccctgagcaaagaccccaacgagaagcgcgatcacatggtcctgctggagttcgtgaccgccgccgggatcactctcggcatggacgagctgtacaagtaacctaggtaccgcggccgcgatccagacatgataagatacattgatgagtttggacaaaccacaactagaatgcagtgaaaaaaatgctttatttgtgaaatttgtgatgctattgctttatttgtaaccattataagctgcaataaacaagttaacaacaacaattgcattcattttatgtttcaggttcagggggaggtgtgggaggttttttaaagcaagtaattgctgggcctttttcccatgcctgcctttactctgccagagttatattgctggggttttgaagaagatcctattaaataaaagaataagcagtattattaagtagccctgcatttcaggtttccttgagtggcaggccaggcctggccgtgaacgttcactgaaatcatggcctcttggccaagattgatagcttgtgcctgtccctgagtcccagtccatcacgagcagctggtttctaagatgctatttcccgtataaagcatgagaccgtgacttgccagccccacagagccccgcccttgtccatcactggcatctggactccagcctgggttggggcaaagagggaaatgagatcatgtcctaaccctgatcctcttgtcccacagatatccagaaccctgaccctgccgtgtaccagctgagagactctaaatccagtgacaagtctgtctgcctattcaccgattttgattctcaaacaaatgtgtcacaaagtaaggattctgatgtgtatatcacagacaaaactgtgctagacatgaggtctatggacttcaagagcaacagtgctgtggcctggagcaacaaatctgactttgcatgtgcaaacgccttcaacaacagcattattccagaagacaccttcttccccagcccaggtaaggggaattgatggagttggccactccctctctgcgcgctcgctcgctcactgaggccgcccgggcaaagcccgggcgtcgggcgacctttggtcgcccggcctcagtgagcgagcgagcgcgcagagagggagtgg

SEQ ID NO: 66 - DNA, 3262 bp, Artificial Sequence
  Synthesized
gttggccactccctctctgcgcgctcgctcgctcactgaggccgggcgaccaaaggtcgcccgacgcccgggctttgcccgggcggcctcagtgagcgagcgagcgcgcagagagggagtggccaactccatcactaggggttcctacgcgtccagcagctcctgctttctgagggtgaaggatagacgctgtggctctgcatgactcactagcactctatcacggccatattctggcagggtcagtggctccaactaacatttgtttggtactttacagtttattaaatagatgtttatatggagaagctctcatttctttctcagaagagcctggctaggaaggtggatgaggcaccatattcattttgcaggtgaaattcctgagatgtaaggagctgctgtgacttgctcaaggccttatatcaagtaaacggtagcgctggggcttagacgcaggtgttctgatttatagttcaaaacctctatcaatgagagagcaatctcctggtaatgtgatagatttcccaacttaatgccaacataccataaacctcccattctgctaatgcccagcctaagttggggagaccactccagattccaagatgtacagtttgctttgccttgtcgagacagagaagactcttgcgtttctgataggcacctattggtcttactgacatccactttgcctttctctccacaggcggcggtggcgagggcagaggaagtcttctaacatgcggtgacgtggaggagaatcccggccccatggcgctcccagtgacagccttacttttacctctggcgttattattgcacgcggctcgtcctgacatacagatgactcagactacctcttccctatctgcttctttaggcgaccgagtaacaatatcttgccgggccagccaggacatctcaaaatacttaaactggtatcagcagaagccggacggaacagttaagttgctcatttaccacacgtcgagattacactcaggcgttcctagccgattttcgggttccggttccggtacggactacagcctgacaatcagtaaccttgagcaggaggacatcgccacctacttctgtcagcagggcaacacgctcccgtacacattcggtgggggaactaagctggagattaccggaggcggtggcagcggtggcggcggcagcgggggtggcggctcggaggtcaagttacaggagagcggaccgggcttggtcgcacctagccagagcctctcagtcacgtgcactgtgtctggagtcagtctcccagactacggggtatcatggatacgacagccgcctagaaagggcttagagtggctgggggttatctggggaagtgaaaccacatactacaactcagctctcaagagccgcctcaccatcattaaggacaacagtaagtcgcaggttttcttaaagatgaactctctccagactgacgacaccgctatttactactgcgcgaagcactactactacggcgggagttacgcaatggactactggggtcagggcacttctgtgaccgtatccagcactactaccccagccccacgtccccccacgccagctccaacgatagcaagtcagcccttatctcttcgccctgaggcttgcaggcccgcggcgggcggcgccgttcacacgcgaggactagacttcgcctgcgacatctacatctgggcaccactagccgggacttgcggagtgttgttgttgagcttggtaataacgctctactgcaaagcgagccgcaaaaaagcggcggcggcggcgaaaagcccgtttgcgagcccggcgagcagcgcgcaggaagaagatgcgagcagctgccgcgcgccgagcgaagaagaaggcagctgcgaactgagagtgaagttctctcgctccgcggacgcacccgcttaccagcagggtcagaaccagctatacaacgagttaaacctggggcgccgggaggagtacgacgtgttagacaagcgtagaggtagggacccggagatgggaggcaagcctcggagaaagaacccccaggagggcctgtacaacgaactccagaaggacaagatggctgaggcgtactcggagattggtatgaagggcgagagacgtcgcggaaagggacacgacggcttataccaggggctttccaccgcgaccaaggacacatacgacgcgctgcacatgcaagccttaccacctcgatgaggtaccagcggccgcgatccagacatgataagatacattgatgagtttggacaaaccacaactagaatgcagtgaaaaaaatgctttatttgtgaaatttgtgatgctattgctttatttgtaaccattataagctgcaataaacaagttaacaacaacaattgcattcattttatgtttcaggttcagggggaggtgtgggaggttttttaaagcaagtaattgctgggcctttttcccatgcctgcctttactctgccagagttatattgctggggttttgaagaagatcctattaaataaaagaataagcagtattattaagtagccctgcatttcaggtttccttgagtggcaggccaggcctggccgtgaacgttcactgaaatcatggcctcttggccaagattgatagcttgtgcctgtccctgagtcccagtccatcacgagcagctggtttctaagatgctatttcccgtataaagcatgagaccgtgacttgccagccccacagagccccgcccttgtccatcactggcatctggactccagcctgggttggggcaaagagggaaatgagatcatgtcctaaccctgatcctcttgtcccacagatatccagaaccctgaccctgccgtgtaccagctgagagactctaaatccagtgacaagtctgtctgcctattcaccgattttgattctcaaacaaatgtgtcacaaagtaaggattctgatgtgtatatcacagacaaaactgtgctagacatgaggtctatggacttcaagagcaacagtgctgtggcctggagcaacaaatctgactttgcatgtgcaaacgccttcaacaacagcattattccagaagacaccttcttccccagcccaggtaaggggaattgatggagttggccactccctctctgcgcgctcgctcgctcactgaggccgcccgggcaaagcccgggcgtcgggcgacctttggtcgcccggcctcagtgagcgagcgagcgcgcagagagggagtgg